European Patent Specification EP 3 763 825 B1, published October 4, 2023. Title: HIGH MULTIPLEX PCR WITH MOLECULAR BARCODING. Applicant: Qiagen Sciences, LLC Wang, Yexun Peng, Quan. Application PCT. The sequence listing filed with the application follows.

SEQUENCE LISTING (8 sequences)

SEQ ID NO: 1 - DNA, 48 bp, Artificial Sequence
  Exemplary BC primer
  misc_feature (1)...(48): n = A,T,C or G
aatgtacagtattgcgttttgnnnnnnnnnncggcaggagacgaagag

SEQ ID NO: 2 - DNA, 21 bp, Artificial Sequence
  BC primer sequence
aatgtacagtattgcgttttg

SEQ ID NO: 3 - DNA, 17 bp, Artificial Sequence
  BC primer sequence
cggcaggagacgaagag

SEQ ID NO: 4 - DNA, 38 bp, Artificial Sequence
  Exemplary LA primer
ttcttagcgtattggagtccaaagccgaggaagctttg

SEQ ID NO: 5 - DNA, 20 bp, Artificial Sequence
  LA primer sequence
ttcttagcgtattggagtcc

SEQ ID NO: 6 - DNA, 18 bp, Artificial Sequence
  LA primer sequence
aaagccgaggaagctttg

SEQ ID NO: 7 - DNA, 79 bp, Artificial Sequence
  Universal adapter primers, Uni.Primer1
aatgatacggcgaccaccgagatctacactctttccctacacgacgctcttccgatctaatgtacagtattgcgttttg

SEQ ID NO: 8 - DNA, 84 bp, Artificial Sequence
  Universal adapter primers, Uni.Primer2
caagcagaagacggcatacgagatacatcggtgactggagttcagacgtgtgctcttccgatctttcttagcgtattggagtcc